European Patent Specification EP 3 842 412 B1, published April 24, 2024. Title: Biodegradable Compound, Lipid Particle, Composition Comprising Lipid Particle, and Kit. Applicant: KABUSHIKI KAISHA TOSHIBA. The sequence listing filed with the application follows.

SEQUENCE LISTING (2 sequences)

SEQ ID NO: 1 - protein, 20 aa, Artificial Sequence
  mHP-1
RQRQRYYRQRQRGGRRRRRR

SEQ ID NO: 2 - protein, 21 aa, Artificial Sequence
  mHP-2
RRRRRRYYRQRQRGGRRRRRR